European Patent Application EP 4 574 964 A1, published June 25, 2025. Title: 신규 유산균 및 이의 용도. Applicant: PBLbiolab. Application KR. The sequence listing filed with the application follows.

SEQUENCE LISTING (6 sequences)

SEQ ID NO: 1 - DNA, 780 bp, Lactococcus lactis
  source 1..780: mol_type = other DNA
tggctcaggacgaacgctggcggcgtgcctaatacatgcaagttgagcgctgaaggttggtacttgtaccaactggatgagcagcgaacgggtgagtaacgcgtggggaatctgcctttgagcgggggacaacatttggaaacgaatgctaataccgcataaaaactttaaacacaagttttaagtttgaaagatgcaattgcatcactcaaagatgatcccgcgttgtattagctagttggtgaggtaaaggctcaccaaggcgatgatacatagccgacctgagagggtgatcggccacattgggactgagacacggcccaaactcctacgggaggcagcagtagggaatcttcggcaatggacgaaagtctgaccgagcaacgccgcgtgagtgaagaaggttttcggatcgtaaaactctgttggtagagaagaacgttggtgagagtggaaagctcatcaagtgacggtaactacccagaaagggacggctaactacgtgccagcagccgcggtaatacgtaggtcccgagcgttgtccggatttattgggcgtaaagcgagcgcaggtggtttattaagtctggtgtaaaaggcagtggctcaaccattgtatgcattggaaactggtagacttgagtgcaggagaggagagtggaattccatgtgtagcggtgaaatgcgtagatatatggaggaacaccggtggcgaaagcggctctctggcctgtaactgacactgaggctcgaaagcgtggggagcaaacaggattagat

SEQ ID NO: 2 - DNA, 780 bp, Bifidobacterium bifidum
  source 1..780: mol_type = other DNA
tatggctcaggatgaacgctggcggcgtgcttaacacatgcaagtcgaacgggatccatcaagcttgcttggtggtgagagtggcgaacgggtgagtaatgcgtgaccgacctgccccatgctccggaatagctcctggaaacgggtggtaatgccggatgttccacatgatcgcatgtgattgtgggaaagatttcatcggcgtgggatggggtcgcgtcctatcagcttgttggtgaggtaacggctcaccaaggcttcgacgggtagccggcctgagagggcgaccggccacattgggactgagatacggcccagactcctacgggaggcagcagtggggaatattgcacaatgggcgcaagcctgatgcagcgacgccgcgtgagggatggaggccttcgggttgtaaacctcttttgtttgggagcaagccttcgggtgagtgtacctttcgaataagcgccggctaactacgtgccagcagccgcggtaatacgtagggcgcaagcgttatccggatttattgggcgtaaagggctcgtaggcggctcgtcgcgtccggtgtgaaagtccatcgcttaacggtggatctgcgccgggtacgggcgggctggagtgcggtaggggagactggaattcccggtgtaacggtggaatgtgtagatatcgggaagaacaccgatggcgaaggcaggtctctgggccgtcactgacgctgaggagcgaaagcgtggggagcgaacaggattagataccctggtagtccacgccgtaaac

SEQ ID NO: 3 - DNA, 22 bp, synthetic construct
  source 1..22: mol_type = other DNA
ttactggtgtatcactgtaagg

SEQ ID NO: 4 - DNA, 19 bp, synthetic construct
  source 1..19: mol_type = other DNA
ccgtcacaggctgaacagt

SEQ ID NO: 5 - DNA, 21 bp, synthetic construct
  source 1..21: mol_type = other DNA
acggtcttgctgtcacttata

SEQ ID NO: 6 - DNA, 24 bp, synthetic construct
  source 1..24: mol_type = other DNA
tacacatatgttcttccctaataa